European Patent Application EP 4 321 535 A1, published February 14, 2024. Title: ANTI-CNTN4 ANTIBODY AND ITS USE. Applicant: GENOME AND COMPANY. The sequence listing filed with the application follows.

SEQUENCE LISTING (159 sequences)

SEQ ID NO: 1 - protein, 101 aa, Artificial Sequence
  S1 VL
ALTQPSSVSANPGETVKITCSGGSSYGWYQQKSPGSAPVTVIYDNTNRPSNIPSRFSGSKSGSTNTLTITGVRAEDEAVYFCGGYDSSIDAFGAGTTLTVL

SEQ ID NO: 2 - protein, 123 aa, Artificial Sequence
  S1,S2,S3,S6,S129,S130,S131,S134,S135,S137,S138,A-01 VH
AVTLDESEGGLQTPGGALSLVCKASGFTFSSFNMFWVRQAPGKGLEYVAEISGGGGSTWYAPAVKGRATISRDNGQSTVRLQLNNLRAEDTGTYYCAKSADTWSYGAATIDAWGHGTEVIVSS

SEQ ID NO: 3 - protein, 104 aa, Artificial Sequence
  S2,S130,S132 VL
ALTQPSSVSANPGETVKITCSGGGSSTYYGWYQQKSPGSAPVTVIYNNNNRPSDIPSRFSGSGSGSTGTLTITGVRAEDEAVYYCGGYDGSTDVFGAGTTLTVL

SEQ ID NO: 4 - protein, 101 aa, Artificial Sequence
  S3 VL
ALTQPSSVSANPGETVKITCSGGSSYGWYQQKAPGSAPVTLIYDNTNRPSNIPSRFSGSTSGSTGTLTITGVRAEDEAVYFCGGYDGSTDAFGAGTTLTVL

SEQ ID NO: 5 - protein, 103 aa, Artificial Sequence
  S4 VL
ALTQPSSVSANPGESVKITCSGGGSSYYGWYQQKSPGSAPVTLIYQNTNRPSNIPSRFSGSGSGSTGTLTITGVRAEDEAVYYCGGYDGSTDVFGAGTTLTVL

SEQ ID NO: 6 - protein, 123 aa, Artificial Sequence
  S4 VH
AVTLDESEGGLQTPGGALSLVCKASGFTFSSFNMFWVRQAPGKGLEYVAEISGGGGSTWYASAVKGRATISRDNGQSTVRLQLNNLRAEDTGTYYCAKSADTWSYGAATIDAWGHGTEVIVSS

SEQ ID NO: 7 - protein, 102 aa, Artificial Sequence
  S6 VL
ALTQPSSVSANPGETVKITCSGGSGNYGWYQQKSPGSAPVTVIYNGNNRPSDIPSRFSGSGSGSTNTLAITGVQAEDEAVYFCGGYDGTIDAFGAGTTLTVL

SEQ ID NO: 8 - protein, 102 aa, Artificial Sequence
  S7,S8,S9,S10,S11,S15,S24,S30 VL
ALTQPSSVSANPGETVEITCSGGSGSYGWYQQKAPGSAPVTVIYDNTNRPSNIPSRFSGSGSDSTGTLTITGVQADDEAVYYCGSYDSIEVIFGAGTTLTVL

SEQ ID NO: 9 - protein, 124 aa, Artificial Sequence
  S7,S8,S9,S10,S11,S15,S30,S46,A13WB2,A13WB4,A13WB7,A13WB24,A13WB25 ,A13SF7,A13SF8,A13SF20,A13SF21,A35WB1,A35WB27,A35SF5,A35SF8,A35SF 13,A35SF14,A35SF37,A35SF38,A35SF39,A35SF75,A35SF90 VH
AVTLDESGGGLHTPGGALSLVCKASGFTFSSYGMAWVRQAPGKGLEWVAGITSSGSSAGYGPAVKGRATISRDNGQSTVRLQLNNLRAEDTATYYCAKDGYIYSGADSDSIDAWGHGTEVIVSS

SEQ ID NO: 10 - protein, 124 aa, Artificial Sequence
  S24 VH
AVTLDESGGGLHTPGGALSLVCKASGFTFSSYGMAWVRQAPGKGLEWVAGITSSGSSAGYGPAVKGRATISRDNGQSTVRLQLNNLRAEDTATYYCAKDGYIYSGGDSDSIDAWGHGTEVIVSS

SEQ ID NO: 11 - protein, 102 aa, Artificial Sequence
  S46 VL
ALTQPSSVSANPGETVEITCSGGSGSYGWYQQKAPGSAPVTVIYDNTNRPSNIPSRFSGSGSDSTGTLTITGVQADDKAVYYCGSYDSIEVIFGAGTTLTVL

SEQ ID NO: 12 - protein, 109 aa, Artificial Sequence
  S83 VL
ALTQPSSVSANLGETVKITCSGGGGYSGSYYYGWYQQKSPAGAPDTVIYSNNQRPSNIPSRFSGSKSGSTGTLTITEDHAEDEAVYYCGSIDSSSNPGIFGAGTTLTVL

SEQ ID NO: 13 - protein, 125 aa, Artificial Sequence
  S83 VH
AVTLDKSGGGLHTPGGALSLVCKASGFTFSRYIMQWVLQAPGKVLEWVASIRNGTTPKYGAAVKGRATISRDNGQSTVMLQLNSLTYDDTDAYYCDRGDDGDCICGGCAASIDIWCYATEVIVSS

SEQ ID NO: 14 - protein, 105 aa, Artificial Sequence
  S96 VL
ALTQPSSVSANPGETVKITCSGSSGSYGYSWHQQKSPGSAPVTVIYESNKRPSNIPSRFSGSTSGSTSTLTITGVQADDEAVYFCGSADSSTTIAFGAGTTLTVL

SEQ ID NO: 15 - protein, 124 aa, Artificial Sequence
  S96 VH
AVTLDESGGGLQTPGGTLSLVCKASGFTFSTYSMQWLRQAPGKGLEWVAGISNSGSSTVYGPAVKGRATISRDNGQSTVSLQLNNLRAEDTGTYYCAKSTYGGSWYAAYSIDEWGHGTEVIVSS

SEQ ID NO: 16 - protein, 110 aa, Artificial Sequence
  S99 VL
ALTQPSSVSANPGETVKITCSGGASYAGNYYYGWYQQKSPGSAPVTVIYNNNQRPSDIPSRFSGSLSGSTNTLTITGVQADDEAVYFCGSDDSSAGYTGIFGAGTTLTVL

SEQ ID NO: 17 - protein, 127 aa, Artificial Sequence
  S99 VH
AVTLDESGGGLQTPGGALSLVCKASEFTFSGYGMHWVRQAPGKGLEFVAEISNTGSWTGYGAAVKGRATISRDNGQSTVRLQLNNLKADDTATYYCAKVGGRGWCGRSGCADDIDAWGHGTEVIVSS

SEQ ID NO: 18 - protein, 102 aa, Artificial Sequence
  S129,A-01 VL
ALTQPSSVSANLGETVKITCSGSSGSYGWYQQKSPGSAPVTLIYDNTNRPSDIPSRFSGSGSGSTGTLTITGVRAEDEAVYYCGGYDGSTDVFGAGTTLTVL

SEQ ID NO: 19 - protein, 103 aa, Artificial Sequence
  S131 VL
ALTQPSSVSANLGGTVKITCSGGGSSYYGWYQQKSPGSAPVTLIYQNTNRPSNIPSRFSGSGSGSTGTLTITGVRAEDEAVYYCGGYDGSTDVFGAGTTLTVL

SEQ ID NO: 20 - protein, 123 aa, Artificial Sequence
  S132 VH
AVTLDESGGGLQTPGGALSLVCKASGFTFSSFNMFWVRQAPGKGLEYVAEISGGGGSTWYAPAVKGRATISRDNGQSTVRLQLNNLRAEDTGTYYCAKSADTWSYGAATIDAWGHGTEVIVSS

SEQ ID NO: 21 - protein, 107 aa, Artificial Sequence
  S134 VL
ALTQPSSVSANPGETVKITCSGGTYSYGNYYYGWYQQKSPGSAPVTVIYNNNNRPSDIPSRFSGSGSGSTGTLTITGVRAEDEAVYYCGGYDGSTDVFGAGTTLTVL

SEQ ID NO: 22 - protein, 103 aa, Artificial Sequence
  S135 VL
ALTQPSSVSANPGETVKITCSGGGSSSYYGWYQQKSPGSAPVTVIYYNNRPSDIPSRFSGSGSGSTGTLTITGVRAEDEAVYYCGGYDGSTDVFGAGTTLTVL

SEQ ID NO: 23 - protein, 101 aa, Artificial Sequence
  S137 VL
ALTQPSSVSANPGETVKITCSGGSSYGWYQQKSPGSAPVTVIYDNTNRPSNIPSRFSGSKSGSTNTLTITGVQAEDEAVYYCGGYDGSTDAFGAGTTLTVL

SEQ ID NO: 24 - protein, 107 aa, Artificial Sequence
  S138 VL
ALTQPSSVSANPGETVNITCSGGGSYAGSYYYGWYQQKAPGSAPVTVIYDSTNRPSNIPSRFSGSLSGSTNTLTITGVRAEDEAVYYCGGYDGSTDVFGAGTTLTVL

SEQ ID NO: 25 - protein, 104 aa, Artificial Sequence
  A13WB2 VL
ALTQPSSVSANLGGTVEITCSGGYSGYGWYQQKSPGSAPVTLIYYNDKRPSDIPSRFSGSKSGSTGTLTITGVQAEDEAVYFCGSRDSSTYVDIFGAGTTLTVL

SEQ ID NO: 26 - protein, 107 aa, Artificial Sequence
  A13WB4 VL
ALTQPSSVSANPGETVEITCSGGSSDYGYGWYQQKSPGSAPVTVIYYNNNRPSDIPSRFSGSLSGSTNTLTITGVQADDEAVYFCGSRDSSSGYVDIFGAGTTLTVL

SEQ ID NO: 27 - protein, 108 aa, Artificial Sequence
  A13WB7 VL
ALTQPSSVSANPGETVKITCSGGGSSSYYNYGWYQQKSPGSAPVTVIYYNDKRPSDIPSRFSGSKSGSTGTLTITGVQAEDEAVYYCGSWDSSTYSDIFGAGTTLTVL

SEQ ID NO: 28 - protein, 104 aa, Artificial Sequence
  A13WB24 VL
ALTQPSSVSANPGGTVEITCSGGGNNNYGWYQQKSPGSAPVTLIYYNDNRPSDIPSRFSGSKSGSTATLTITGVQAEDEAVYYCGGYDISYVDIFGAGTTLTVL

SEQ ID NO: 29 - protein, 104 aa, Artificial Sequence
  A13WB25 VL
ALTQPSSVSANLGGTVEITCSGGGGSYGWYQQKSPGSAPVTVIYYNDKRPSDIPSRFSGSKSGSTGTLTITGVQAEDEAVYFCGGYDGSTYAGIFGAGTTLTVL

SEQ ID NO: 30 - protein, 104 aa, Artificial Sequence
  A13WB73 VL
ALTQPSSVSANLGGTVEITCSGGYSGYGWYQQMSPGSAPVTLTYYNDKRPSNIPSRFSGSKSGSTATLAITGVQAEDEAVYYCGSWDTSTNTPIFGAGTTLTVL

SEQ ID NO: 31 - protein, 124 aa, Artificial Sequence
  A13WB73 VH
AVTLDESGGGLHTPGGVLSLVCKASGFTFSSYGMAWVRQAPGKGLEWVAGITSSGSSAGYGPAVKGRATISRDNGQSTVRLQLNNLRAEDTATYYCAKDGYIYSGADSDSIDAWGHGTEVIVSS

SEQ ID NO: 32 - protein, 104 aa, Artificial Sequence
  A13SF1 VL
ALTQPSSVSANLGGTVKITCSGGGGSYGWFQQKSPGSAPVTLIYNNNNRPSDIPSRFSGSKSGSTATLTITGVQAEDEAVYFCGGYDSSTYVGTFGAGTTLTVL

SEQ ID NO: 33 - protein, 124 aa, Artificial Sequence
  A13SF1,A13SF16,A35SF3 VH
AVTLDESGGGLQTPGGGLSLVCKASGFTFSSYGMAWVRQAPGKGLEWVAGITSSGSSAGYGPAVKGRATISRDNGQSTVRLQLNNLRAEDTATYYCAKDGYIYSGADSDSIDAWGHGTEVIVSS

SEQ ID NO: 34 - protein, 105 aa, Artificial Sequence
  A13SF2 VL
ALTQPSSVSANLGGTVKITCSGGGGSYGWYRQKSPGSAPVTLIYNNNNRPSDIPSRFSGSTSGSTGTLTITGVQADDEAVYFCGGYDSSAGYAALFGAGTTLTVL

SEQ ID NO: 35 - protein, 124 aa, Artificial Sequence
  A13SF2 VH
AVTLDESGGGLQTPGGALSLICKASGFTFSSYGMAWVRQAPGKGLEWVAGITSSGSSAGYGPAVKGRATISRDNGQSTVRLQLNNLRAEDTATYYCAKDGYIYSGADSDSIDAWGHGTEVIVSS

SEQ ID NO: 36 - protein, 105 aa, Artificial Sequence
  A13SF7 VL
ALTQPSSVSANLGGTVEITCSGGSGSYGWYQQKSPGSAPVTLIYDNTNRPSNIPSRFSGSTSGSTSTLTITGVQADDEAVYFCGSADTNAAYAAIFGAGTTLTVL

SEQ ID NO: 37 - protein, 103 aa, Artificial Sequence
  A13SF8 VL
ALTQPSSVSANPGGTVKITCSGSGNYGWYQQKSPGSALVTVIYYNDKRPSDIPSRFSGSTSGSTGTLTITGVQVEDEAVYYCGGYDGYSFASIFGAGTTLTVL

SEQ ID NO: 38 - protein, 104 aa, Artificial Sequence
  A13SF16 VL
ALTQPSSVSANLGGTVKITCSGSGGSYGWFQQKSPGSAPVTLIYNNDNRPSDIPSRFSGSKSGSTATLTITGVQAEDEAVYFCGGYDSSTYVDTFGAGTTLTVL

SEQ ID NO: 39 - protein, 105 aa, Artificial Sequence
  A13SF19 VL
ALTQPSSVSANLGGTVEITCSGSSSGNYGWYQQKSPGSAPVTVIYYNDERPSDIPSRFSGSKSGSTGTLTITGVQAEDEAVYYCGGYEGSTYVGIFGAGTTLTVL

SEQ ID NO: 40 - protein, 124 aa, Artificial Sequence
  A13SF19 VH
AVTLDESGGGLHTPGGALSLVCKASGFTFSSYGMAWVRQASGKGLEWVAGITSSGSSAGYGPAVKGRATISRDNGQSTVRLQLNNLRAEDTATYYCAKDGYIYSGADSDSIDAWGHGTEVIVSS

SEQ ID NO: 41 - protein, 101 aa, Artificial Sequence
  A13SF20 VL
ALTQPSSVSANLGGTVEITCSGGSGSYGWYQQKAPGSAPVTLIYNSDKRPSDIPSRFSGSKSGSTGTLTITGVQAEDEAVYFCGGYDSSAIFGAGTTLTVL

SEQ ID NO: 42 - protein, 104 aa, Artificial Sequence
  A13SF21 VL
ALTQPSSVSANLGGTVEITCSGSSGSYGWYQQKAPGSAPVTVIYNNNNRPSGIPSRFSGALSGSTATLTITGVQAEDEAVYFCGGYDSSTYVGIFGAGTTLTVL

SEQ ID NO: 43 - protein, 106 aa, Artificial Sequence
  A13SF74 VL
ALTQPSSVSANPGETVKITCSGNSSGCSWYGWFQQKSPGSALVTVIYDNTNRPSNIPSRFSGSRSGSTATLTITGVQAEDEAIYFCGIADSSGAGIFGAGTTLTVL

SEQ ID NO: 44 - protein, 123 aa, Artificial Sequence
  A13SF74 VH
AVTLDESGGGLQTPGGALSLVCKASGFTLSSYAMQWVRQAPGKGLEWVAGISKGGGSTAYGAAVKGRATISRDNGQSTVRLQLNNLRAEDTATYFCAKTTDSNCCSSDSIDAWGHGTEVIVSS

SEQ ID NO: 45 - protein, 103 aa, Artificial Sequence
  A35WB1 VL
ALTQPSSVSANPGETVKITCSGGSGSYGWYQQKSPGSAPVTVIYNNDQRPSNIPSRFSGSKSGSTATLTITGVQVEDEAVYFCGGWDSNSGAIFGAGTTLTVL

SEQ ID NO: 46 - protein, 105 aa, Artificial Sequence
  A35WB27 VL
ALTQPSSVSANLGETVKITCSGGYSGYGWYQQKSPGSAPVTVIYYNDKRPSDIPSRFSGSKSGSTGTLTITGVRAEDEAVYFCGSADSSTGYVAIFGAGTTLTVL

SEQ ID NO: 47 - protein, 101 aa, Artificial Sequence
  A35SF3 VL
ALTQPSSVSANLGGTVEITCSGSSGSYGWYQQKAPGSAPVTVIYDNTNRPSDIPSRFSGSKSGSTGTLTITGVQAEDEAVYFCGGYDSSTIFGAGTTLTVL

SEQ ID NO: 48 - protein, 105 aa, Artificial Sequence
  A35SF5 VL
ALTQPSSVSANPGETVEITCSGSSGSNYGWYQQKSPGSAPVTLIYYNDNRPSDIPSRFSGSKSGSTGTLTITGVQVEDEAVYYCGAWESSSNPDIFGAGTTLTVL

SEQ ID NO: 49 - protein, 104 aa, Artificial Sequence
  A35SF8 VL
ALTQPSSVSANLGGTVKITCSGGGGSYGWFQQKSPGSAPVTLIYNNNNRPSDIPSRFSGSKSGSTATLTITGVQAEDEAVYFCGGYDDSTYVGMFGAGTTLTVL

SEQ ID NO: 50 - protein, 104 aa, Artificial Sequence
  A35SF13 VL
ALTQPSSVSANPGETVKITCSGGGGSYGWYQQKSPGSALVTVIYNNDNRPSNIPSRLSGSKSGSTATLTITGVRAEDEAVYFCGSADNNGYIAIFGAGTTLTVL

SEQ ID NO: 51 - protein, 104 aa, Artificial Sequence
  A35SF14 VL
ALTQPSSVSANPGETIKITCSGGGGSYGWYQQKSPGSAPVTVIYNGNNRPSDIPSRFSGSKSGSTATLTITGVQAEDEAVYFCGGYDSGTYSGIFGAGTTLTVL

SEQ ID NO: 52 - protein, 104 aa, Artificial Sequence
  A35SF37 VL
ALTQPSSVSANLGGTVKITCSGGSNNYGWYQQKSPGSAPVTVIYYNNKRPSDIPSRFSGSKSGSTATLTITGVQAEDEAVYFCGGYDSSSNSDVYGAGTTLTVL

SEQ ID NO: 53 - protein, 104 aa, Artificial Sequence
  A35SF38 VL
ALTQPSSVSANLGGTVKLTCSGSSGSYGWYQQKSPGSAPVTLIYNNNNRPSDIPSRFSGSTSGSTGTLTITGVRAEDEAVYFCGGYDSSTYVAIFGAGTTLTVL

SEQ ID NO: 54 - protein, 102 aa, Artificial Sequence
  A35SF39 VL
ALTQPSSVSANLGGTVKITCSGGSGSYGWYQQKSPGSAPVTVIYNNNNRPSDIPSRFSGSTSGSTGTLTITGVRAEDEAVYFCGGYDTDSPIFGAGTTLTVL

SEQ ID NO: 55 - protein, 104 aa, Artificial Sequence
  A35SF75 VL
ALTQPSSVSANPGVTVKITCSGGGGSYGWYQQKAPGSAPVTLIYNNTNRPSDIPSRFSGSRSGSTNTLTITGVQAEDEAVYFCGGYDSNTDYVGFGAGTTLTVL

SEQ ID NO: 56 - protein, 105 aa, Artificial Sequence
  A35SF90 VL
ALTQPSSVSANLGGTVEITCSGSNNNNYGWYQQKTPGSAPVTLIYNNNQRPSDIPSRFSGSKSGSTGTLTITGVRAEDEAVYYCGGYDSSIYFDIFGAGTTLTVL

SEQ ID NO: 57 - protein, 5 aa, Artificial Sequence
  S1,S3,S137 VL CDR1
SGGSS

SEQ ID NO: 58 - protein, 5 aa, Artificial Sequence
  S1,S2,S3,S4,S6,S129,S130,S131,S132,S134,S135,S137,S138 VH CDR1
SFNMF

SEQ ID NO: 59 - protein, 8 aa, Artificial Sequence
  S2,S130,S132 VL CDR1
SGGGSSTY

SEQ ID NO: 60 - protein, 7 aa, Artificial Sequence
  S4, S131 VL CDR1
SGGGSSY

SEQ ID NO: 61 - protein, 6 aa, Artificial Sequence
  S6 VL CDR1
SGGSGN

SEQ ID NO: 62 - protein, 6 aa, Artificial Sequence
  S7,S8,S9,S10,S11,S15,S24,S30,S46,A13SF20,A35 WB1,A35SF39 VL CDR1
SGGSGS

SEQ ID NO: 63 - protein, 5 aa, Artificial Sequence
  S7~11,S15,S24,S30,S46,A13WB2,A13WB4,A13WB7,A13WB24,A13WB25,A13WB7 3,A13SF1,A13SF2,A13SF7,A13SF8,A13SF16,A13SF19,A13S F20,A13SF21,A35WB1,A35WB27,A35SF3,A35SF5,A35SF8,A35SF13,A35SF14,A 35SF37,A35SF38,A35SF39,A35SF75,A35SF90 VH CDR1
SYGMA

SEQ ID NO: 64 - protein, 11 aa, Artificial Sequence
  S83 VL CDR1
SGGGGYSGSYY

SEQ ID NO: 65 - protein, 5 aa, Artificial Sequence
  S83 VH CDR1
RYIMQ

SEQ ID NO: 66 - protein, 8 aa, Artificial Sequence
  S96 VL CDR1
SGSSGSYG

SEQ ID NO: 67 - protein, 5 aa, Artificial Sequence
  S96 VH CDR1
TYSMQ

SEQ ID NO: 68 - protein, 11 aa, Artificial Sequence
  S99 VL CDR1
SGGASYAGNYY

SEQ ID NO: 69 - protein, 5 aa, Artificial Sequence
  S99 VH CDR1
GYGMH

SEQ ID NO: 70 - protein, 6 aa, Artificial Sequence
  S129,A13SF21,A35SF3,A35SF38 VL CDR1
SGSSGS

SEQ ID NO: 71 - protein, 11 aa, Artificial Sequence
  S134 VL CDR1
SGGTYSYGNYY

SEQ ID NO: 72 - protein, 7 aa, Artificial Sequence
  S135 VL CDR1
GGGSSSY

SEQ ID NO: 73 - protein, 11 aa, Artificial Sequence
  S138 VL CDR1
SGGGSYAGSYY

SEQ ID NO: 74 - protein, 6 aa, Artificial Sequence
  A13WB2,A13WB73,A35WB27 VL CDR1
SGGYSG

SEQ ID NO: 75 - protein, 8 aa, Artificial Sequence
  A13WB4 VL CDR1
SGGSSDYG

SEQ ID NO: 76 - protein, 10 aa, Artificial Sequence
  A13WB7 VL CDR1
SGGGSSSYYN

SEQ ID NO: 77 - protein, 7 aa, Artificial Sequence
  A13WB24 VL CDR1
SGGGNNN

SEQ ID NO: 78 - protein, 6 aa, Artificial Sequence
  A13WB25,A13SF1,A13SF2,A35SF8,A35SF13,A35SF14,A35SF75 VL CDR1
SGGGGS

SEQ ID NO: 79 - protein, 5 aa, Artificial Sequence
  A13SF7 VL CDR1
GGSGS

SEQ ID NO: 80 - protein, 5 aa, Artificial Sequence
  A13SF8 VL CDR1
SGSGN

SEQ ID NO: 81 - protein, 6 aa, Artificial Sequence
  A13SF16 VL CDR1
SGSGGS

SEQ ID NO: 82 - protein, 7 aa, Artificial Sequence
  A13SF19 VL CDR1
SGSSSGN

SEQ ID NO: 83 - protein, 9 aa, Artificial Sequence
  A13SF74 VL CDR1
SGNSSGCSW

SEQ ID NO: 84 - protein, 5 aa, Artificial Sequence
  A13SF74 VH CDR1
SYAMQ

SEQ ID NO: 85 - protein, 7 aa, Artificial Sequence
  A35SF5 VL CDR1
SGSSGSN

SEQ ID NO: 86 - protein, 6 aa, Artificial Sequence
  A35SF37 VL CDR1
SGGSNN

SEQ ID NO: 87 - protein, 7 aa, Artificial Sequence
  A35SF90 VL CDR1
SGSNNNN

SEQ ID NO: 88 - protein, 7 aa, Artificial Sequence
  S1,S3,S7,S8,S9,S10,S11,S15,S24,S30,S46,S129,S137,A13SF7,A13SF74,A 35SF3 VL CDR2
DNTNRPS

SEQ ID NO: 89 - protein, 17 aa, Artificial Sequence
  S1,S2,S3,S6,S129,S130,S131,S132,S134,S135,S137,S138 VH CDR2
EISGGGGSTWYAPAVKG

SEQ ID NO: 90 - protein, 7 aa, Artificial Sequence
  S2,S130,S132,S134,A13SF1,A13SF2,A13SF21,A35SF8,A35SF38,A35SF39 VL CDR2
NNNNRPS

SEQ ID NO: 91 - protein, 7 aa, Artificial Sequence
  S4,S131 VL CDR2
QNTNRPS

SEQ ID NO: 92 - protein, 17 aa, Artificial Sequence
  S4 VH CDR2
EISGGGGSTWYASAVKG

SEQ ID NO: 93 - protein, 7 aa, Artificial Sequence
  S6,A35SF14 VL CDR2
NGNNRPS

SEQ ID NO: 94 - protein, 17 aa, Artificial Sequence
  S7~11,S15,S24,S30,S46,A13WB2,A13WB4,A13WB7,A13WB24,A13WB25,A13WB7 3,A13SF1,A13SF2,A13SF7,A13SF8,A13SF16,A13SF19,A13SF20,A13SF21,A35 WB1,A35WB27,A35SF3,A35SF5,A35SF8,A35SF13,A35SF14,A35SF37,A35SF38, A35SF39,A35SF75,A35SF90 VH CDR2
GITSSGSSAGYGPAVKG

SEQ ID NO: 95 - protein, 7 aa, Artificial Sequence
  S83 VL CDR2
SNNQRPS

SEQ ID NO: 96 - protein, 16 aa, Artificial Sequence
  S83 VH CDR2
SIRNGTTPKYGAAVKG

SEQ ID NO: 97 - protein, 7 aa, Artificial Sequence
  S96 VL CDR2
ESNKRPS

SEQ ID NO: 98 - protein, 17 aa, Artificial Sequence
  S96 VH CDR2
GISNSGSSTVYGPAVKG

SEQ ID NO: 99 - protein, 7 aa, Artificial Sequence
  S99,A35SF90 VL CDR2
NNNQRPS

SEQ ID NO: 100 - protein, 17 aa, Artificial Sequence
  S99 VH CDR2
EISNTGSWTGYGAAVKG

SEQ ID NO: 101 - protein, 6 aa, Artificial Sequence
  S135 VL CDR2
YNNRPS

SEQ ID NO: 102 - protein, 7 aa, Artificial Sequence
  S138 VL CDR2
DSTNRPS

SEQ ID NO: 103 - protein, 7 aa, Artificial Sequence
  A13WB2,A13WB7,A13WB25,A13WB73,A13SF8,A35WB27 VL CDR2
YNDKRPS

SEQ ID NO: 104 - protein, 7 aa, Artificial Sequence
  A13WB4 VL CDR2
YNNNRPS

SEQ ID NO: 105 - protein, 6 aa, Artificial Sequence
  A13WB24 VL CDR2
YNDNRP

SEQ ID NO: 106 - protein, 7 aa, Artificial Sequence
  A13SF16,A35SF13 VL CDR2
NNDNRPS

SEQ ID NO: 107 - protein, 7 aa, Artificial Sequence
  A13SF19 VL CDR2
YNDERPS

SEQ ID NO: 108 - protein, 7 aa, Artificial Sequence
  A13SF20 VL CDR2
NSDKRPS

SEQ ID NO: 109 - protein, 17 aa, Artificial Sequence
  A13SF74 VH CDR2
GISKGGGSTAYGAAVKG

SEQ ID NO: 110 - protein, 7 aa, Artificial Sequence
  A35WB1 VL CDR2
NNDQRPS

SEQ ID NO: 111 - protein, 7 aa, Artificial Sequence
  A35SF5 VL CDR2
YNDNRPS

SEQ ID NO: 112 - protein, 7 aa, Artificial Sequence
  A35SF37 VL CDR2
YNNKRPS

SEQ ID NO: 113 - protein, 7 aa, Artificial Sequence
  A35SF75 VL CDR2
NNTNRPS

SEQ ID NO: 114 - protein, 9 aa, Artificial Sequence
  S1 VL CDR3
GGYDSSIDA

SEQ ID NO: 115 - protein, 14 aa, Artificial Sequence
  S1,S2,S3,S4,S6,S129,S130,S131,S132,S134,S135,S137,S138 VH CDR3
SADTWSYGAATIDA

SEQ ID NO: 116 - protein, 9 aa, Artificial Sequence
  S2,S4,S129,S130,S131,S132,S134,S135,S138 VL CDR3
GGYDGSTDV

SEQ ID NO: 117 - protein, 9 aa, Artificial Sequence
  S3,S137 VL CDR3
GGYDGSTDA

SEQ ID NO: 118 - protein, 9 aa, Artificial Sequence
  S6 VL CDR3
GGYDGTIDA

SEQ ID NO: 119 - protein, 9 aa, Artificial Sequence
  S7,S8,S9,S10,S11,S15,S24,S30,S46 VL CDR3
GSYDSIEVI

SEQ ID NO: 120 - protein, 15 aa, Artificial Sequence
  S7~11,S15,S30,S46,A13WB2,A13WB4,A13WB7,A13WB24,A13WB25,A13WB73,A1 3SF1,A13SF2,A13SF7,A13SF8,A13SF16,A13SF19,A13SF20,A13SF21,A35WB1, A35WB27,A35SF3,A35SF5,A35SF8,A35SF13,A35SF14,A35SF37,A35SF38,A35S F39,A35SF75,A35SF90 VH CDR3
DGYIYSGADSDSIDA

SEQ ID NO: 121 - protein, 15 aa, Artificial Sequence
  S24 VH CDR3
DGYIYSGGDSDSIDA

SEQ ID NO: 122 - protein, 11 aa, Artificial Sequence
  S83 VL CDR3
GSIDSSSNPGI

SEQ ID NO: 123 - protein, 17 aa, Artificial Sequence
  S83 VH CDR3
GDDGDCICGGCAASIDI

SEQ ID NO: 124 - protein, 10 aa, Artificial Sequence
  S96 VL CDR3
GSADSSTTIA

SEQ ID NO: 125 - protein, 15 aa, Artificial Sequence
  S96 VH CDR3
STYGGSWYAAYSIDE

SEQ ID NO: 126 - protein, 12 aa, Artificial Sequence
  S99 VL CDR3
GSDDSSAGYTGI

SEQ ID NO: 127 - protein, 18 aa, Artificial Sequence
  S99 VH CDR3
VGGRGWCGRSGCADDIDA

SEQ ID NO: 128 - protein, 11 aa, Artificial Sequence
  A13WB2 VL CDR3
GSRDSSTYVDI

SEQ ID NO: 129 - protein, 12 aa, Artificial Sequence
  A13WB4 VL CDR3
GSRDSSSGYVDI

SEQ ID NO: 130 - protein, 11 aa, Artificial Sequence
  A13WB7 VL CDR3
GSWDSSTYSDI

SEQ ID NO: 131 - protein, 10 aa, Artificial Sequence
  A13WB24 VL CDR3
GGYDISYVDI

SEQ ID NO: 132 - protein, 11 aa, Artificial Sequence
  A13WB25 VL CDR3
GGYDGSTYAGI

SEQ ID NO: 133 - protein, 11 aa, Artificial Sequence
  A13WB73 VL CDR3
GSWDTSTNTPI

SEQ ID NO: 134 - protein, 11 aa, Artificial Sequence
  A13SF1 VL CDR3
GGYDSSTYVGT

SEQ ID NO: 135 - protein, 12 aa, Artificial Sequence
  A13SF2 VL CDR3
GGYDSSAGYAAL

SEQ ID NO: 136 - protein, 12 aa, Artificial Sequence
  A13SF7 VL CDR3
GSADTNAAYAAI

SEQ ID NO: 137 - protein, 11 aa, Artificial Sequence
  A13SF8 VL CDR3
GGYDGYSFASI

SEQ ID NO: 138 - protein, 11 aa, Artificial Sequence
  A13SF16 VL CDR3
GGYDSSTYVDT

SEQ ID NO: 139 - protein, 11 aa, Artificial Sequence
  A13SF19 VL CDR3
GGYEGSTYVGI

SEQ ID NO: 140 - protein, 8 aa, Artificial Sequence
  A13SF20 VL CDR3
GGYDSSAI

SEQ ID NO: 141 - protein, 11 aa, Artificial Sequence
  A13SF21 VL CDR3
GGYDSSTYVGI

SEQ ID NO: 142 - protein, 10 aa, Artificial Sequence
  A13SF74 VL CDR3
GIADSSGAGI

SEQ ID NO: 143 - protein, 14 aa, Artificial Sequence
  A13SF74 VH CDR3
TTDSNCCSSDSIDA

SEQ ID NO: 144 - protein, 10 aa, Artificial Sequence
  A35WB1 VL CDR3
GGWDSNSGAI

SEQ ID NO: 145 - protein, 12 aa, Artificial Sequence
  A35WB27 VL CDR3
GSADSSTGYVAI

SEQ ID NO: 146 - protein, 8 aa, Artificial Sequence
  A35SF3 VL CDR3
GGYDSSTI

SEQ ID NO: 147 - protein, 11 aa, Artificial Sequence
  A35SF5 VL CDR3
GAWESSSNPDI

SEQ ID NO: 148 - protein, 11 aa, Artificial Sequence
  A35SF8 VL CDR3
GGYDDSTYVGM

SEQ ID NO: 149 - protein, 11 aa, Artificial Sequence
  A35SF13 VL CDR3
GSADNNGYIAI

SEQ ID NO: 150 - protein, 11 aa, Artificial Sequence
  A35SF14 VL CDR3
GGYDSGTYSGI

SEQ ID NO: 151 - protein, 11 aa, Artificial Sequence
  A35SF37 VL CDR3
GGYDSSSNSDV

SEQ ID NO: 152 - protein, 11 aa, Artificial Sequence
  A35SF38 VL CDR3
GGYDSSTYVAI

SEQ ID NO: 153 - protein, 9 aa, Artificial Sequence
  A35SF39 VL CDR3
GGYDTDSPI

SEQ ID NO: 154 - protein, 11 aa, Artificial Sequence
  A35SF75 VL CDR3
GGYDSNTDYVG

SEQ ID NO: 155 - protein, 11 aa, Artificial Sequence
  A35SF90 VL CDR3
GGYDSSIYFDI

SEQ ID NO: 156 - protein, 101 aa, Artificial Sequence
  humanized antibody VL1
ELTQDPAVSVALGQTVRITCSGSSGSYGWYQQKPGQAPVLVIYDNTNRPSGIPDRFSGSSSGNTASLTITGAQAEDEADYYCGGYDGSTDVFGGGTKLTVL

SEQ ID NO: 157 - protein, 123 aa, Artificial Sequence
  humanized antibody VH1
EVQLLESGGGLVQPGGSLRLSCAASGFTFSSFNMFWVRQAPGKGLEWVSEISGGGGSTWYAPAVKGRFTISRDNSKNTLYLQMNSLRAEDTAVYYCAKSADTWSYGAATIDAWGQGTLVTVSS

SEQ ID NO: 158 - protein, 101 aa, Artificial Sequence
  humanized antibody VL2
ELTQDPAVSVALGQTVRITCSGSSGSYGWYQQKPGQAPVTLIYDNTNRPSGIPDRFSGSSSGSTGSLTITGAQAEDEADYYCGGYDGSTDVFGGGTKLTVL

SEQ ID NO: 159 - protein, 123 aa, Artificial Sequence
  humanized antibody VH2
EVQLLESEGGLVQPGGSLRLSCAASGFTFSSFNMFWVRQAPGKGLEWVAEISGGGGSTWYAPAVKGRATISRDNSKNTVYLQMNSLRAEDTAVYYCAKSADTWSYGAATIDAWGQGTLVTVSS